European Patent Application EP 4 814 006 A2, published September 30, 2026. Title: NOVEL BINDING PROTEINS FOR HYALURONIC ACID. Applicant: Navigo Proteins GmbH. The sequence listing filed with the application follows.

SEQUENCE LISTING (10 sequences)

SEQ ID NO: 1 - protein, 200 aa, synthetic construct
  REGION 1..200: note = hyaluronic acid binding protein
VVFHYRPARGRYALNFAEAQQACLEQDAVIASPEQLQAAWEDGLDQCDAGWLSDQTVRYPITTPREPCGGDKDGFPGVRSYGFRDPDETYDVYCFASALEGEVFYLTPPEKLTFEEAAAACRRRGAALAKVGQLYAAWKFGLDDRCDAGWLADGSVRYPIVTPRPRCGGPLPAGVRTVGFFPNQTGFPDPASRFGAYCFR

SEQ ID NO: 2 - protein, 200 aa, synthetic construct
  REGION 1..200: note = hyaluronic acid binding protein
VVFHYRPGSGRYTLNFEEAQQACLEQGAVIASPEQLQAAYEDGLDQCDAGWLSDQTVRYPITTPREPCYGDKDSFPGVRSYGVRDPDETYDVYCFASELEGEVFYLTPPEKLTLEEARAACRRRGARLAKVGQLYAAWKFGLDDRCDAGWLADGSVRYPIVTPRPRCGGPLPAGVRTVYFFPNQTGFPDPASRYGAYCFR

SEQ ID NO: 3 - protein, 97 aa, synthetic construct
  REGION 1..97: note = hyaluronic acid binding protein
GVFHLESPSGKYGLTFDEAREACEAEGATLATYKQLEAAQKAGFHLCSAGWLATGRVAYPTAKPSPNCGSGRVGIVDYGPRPNKSEQWDAYCYRPHA

SEQ ID NO: 4 - protein, 97 aa, synthetic construct
  REGION 1..97: note = hyaluronic acid binding protein
GVYHREAPSGKYGLTYAEAKAVCEFEGGHLATYKQLEAAQKIGFHVCAAGWMAKGRVGYPIVKPGPNCGFGKTGIIDYGIRLNRSERWDAYCYNPHA

SEQ ID NO: 5 - protein, 646 aa, synthetic construct
  REGION 1..646: note = Fusion protein comprising hyaluronic acid binding protein SEQ ID NO:1
SDTGRPFVEMYSEIPEIIHMTEGRELVIPCRVTSPNITVTLKKFPLDTLIPDGKRIIWDSRKGFIISNATYKEIGLLTCEATVNGHLYKTNYLTHRQTNTIIDVVLSPSHGIELSVGEKLVLNCTARTELNVGIDFNWEYPSSKHQHKKLVNRDLKTQSGSEMKKFLSTLTIDGVTRSDQGLYTCAASSGLMTKKNSTFVRVHEKDKTHTCPPCPAPELLGGPSVFLFPPKPKDTLMISRTPEVTCVVVDVSHEDPEVKFNWYVDGVEVHNAKTKPREEQYNSTYRVVSVLTVLHQDWLNGKEYKCKVSNKALPAPIEKTISKAKGQPREPQVYTLPPSRDELTKNQVSLTCLVKGFYPSDIAVEWESNGQPENNYKTTPPVLDSDGSFFLYSKLTVDKSRWQQGNVFSCSVMHEALHNHYTQKSLSLSPGGGGGSGGGGSGGGGSVVFHYRPARGRYALNFAEAQQACLEQDAVIASPEQLQAAWEDGLDQCDAGWLSDQTVRYPITTPREPCGGDKDGFPGVRSYGFRDPDETYDVYCFASALEGEVFYLTPPEKLTFEEAAAACRRRGAALAKVGQLYAAWKFGLDDRCDAGWLADGSVRYPIVTPRPRCGGPLPAGVRTVGFFPNQTGFPDPASRFGAYCFR

SEQ ID NO: 6 - protein, 646 aa, synthetic construct
  REGION 1..646: note = Fusion protein comprising hyaluronic acid binding protein SEQ ID NO: 2
SDTGRPFVEMYSEIPEIIHMTEGRELVIPCRVTSPNITVTLKKFPLDTLIPDGKRIIWDSRKGFIISNATYKEIGLLTCEATVNGHLYKTNYLTHRQTNTIIDVVLSPSHGIELSVGEKLVLNCTARTELNVGIDFNWEYPSSKHQHKKLVNRDLKTQSGSEMKKFLSTLTIDGVTRSDQGLYTCAASSGLMTKKNSTFVRVHEKDKTHTCPPCPAPELLGGPSVFLFPPKPKDTLMISRTPEVTCVVVDVSHEDPEVKFNWYVDGVEVHNAKTKPREEQYNSTYRVVSVLTVLHQDWLNGKEYKCKVSNKALPAPIEKTISKAKGQPREPQVYTLPPSRDELTKNQVSLTCLVKGFYPSDIAVEWESNGQPENNYKTTPPVLDSDGSFFLYSKLTVDKSRWQQGNVFSCSVMHEALHNHYTQKSLSLSPGGGGGSGGGGSGGGGSVVFHYRPGSGRYTLNFEEAQQACLEQGAVIASPEQLQAAYEDGLDQCDAGWLSDQTVRYPITTPREPCYGDKDSFPGVRSYGVRDPDETYDVYCFASELEGEVFYLTPPEKLTLEEARAACRRRGARLAKVGQLYAAWKFGLDDRCDAGWLADGSVRYPIVTPRPRCGGPLPAGVRTVYFFPNQTGFPDPASRYGAYCFR

SEQ ID NO: 7 - protein, 543 aa, synthetic construct
  REGION 1..543: note = Fusion protein comprising hyaluronic acid binding protein SEQ ID NO: 3
SDTGRPFVEMYSEIPEIIHMTEGRELVIPCRVTSPNITVTLKKFPLDTLIPDGKRIIWDSRKGFIISNATYKEIGLLTCEATVNGHLYKTNYLTHRQTNTIIDVVLSPSHGIELSVGEKLVLNCTARTELNVGIDFNWEYPSSKHQHKKLVNRDLKTQSGSEMKKFLSTLTIDGVTRSDQGLYTCAASSGLMTKKNSTFVRVHEKDKTHTCPPCPAPELLGGPSVFLFPPKPKDTLMISRTPEVTCVVVDVSHEDPEVKFNWYVDGVEVHNAKTKPREEQYNSTYRVVSVLTVLHQDWLNGKEYKCKVSNKALPAPIEKTISKAKGQPREPQVYTLPPSRDELTKNQVSLTCLVKGFYPSDIAVEWESNGQPENNYKTTPPVLDSDGSFFLYSKLTVDKSRWQQGNVFSCSVMHEALHNHYTQKSLSLSPGGGGGSGGGGSGGGGSGVFHLESPSGKYGLTFDEAREACEAEGATLATYKQLEAAQKAGFHLCSAGWLATGRVAYPTAKPSPNCGSGRVGIVDYGPRPNKSEQWDAYCYRPHA

SEQ ID NO: 8 - protein, 543 aa, synthetic construct
  REGION 1..543: note = Fusion protein comprising hyaluronic acid binding protein SEQ ID NO: 4
SDTGRPFVEMYSEIPEIIHMTEGRELVIPCRVTSPNITVTLKKFPLDTLIPDGKRIIWDSRKGFIISNATYKEIGLLTCEATVNGHLYKTNYLTHRQTNTIIDVVLSPSHGIELSVGEKLVLNCTARTELNVGIDFNWEYPSSKHQHKKLVNRDLKTQSGSEMKKFLSTLTIDGVTRSDQGLYTCAASSGLMTKKNSTFVRVHEKDKTHTCPPCPAPELLGGPSVFLFPPKPKDTLMISRTPEVTCVVVDVSHEDPEVKFNWYVDGVEVHNAKTKPREEQYNSTYRVVSVLTVLHQDWLNGKEYKCKVSNKALPAPIEKTISKAKGQPREPQVYTLPPSRDELTKNQVSLTCLVKGFYPSDIAVEWESNGQPENNYKTTPPVLDSDGSFFLYSKLTVDKSRWQQGNVFSCSVMHEALHNHYTQKSLSLSPGGGGGSGGGGSGGGGSGVYHREAPSGKYGLTYAEAKAVCEFEGGHLATYKQLEAAQKIGFHVCAAGWMAKGRVGYPIVKPGPNCGFGKTGIIDYGIRLNRSERWDAYCYNPHA

SEQ ID NO: 9 - protein, 431 aa, synthetic construct
  REGION 1..431: note = Aflibercept
SDTGRPFVEMYSEIPEIIHMTEGRELVIPCRVTSPNITVTLKKFPLDTLIPDGKRIIWDSRKGFIISNATYKEIGLLTCEATVNGHLYKTNYLTHRQTNTIIDVVLSPSHGIELSVGEKLVLNCTARTELNVGIDFNWEYPSSKHQHKKLVNRDLKTQSGSEMKKFLSTLTIDGVTRSDQGLYTCAASSGLMTKKNSTFVRVHEKDKTHTCPPCPAPELLGGPSVFLFPPKPKDTLMISRTPEVTCVVVDVSHEDPEVKFNWYVDGVEVHNAKTKPREEQYNSTYRVVSVLTVLHQDWLNGKEYKCKVSNKALPAPIEKTISKAKGQPREPQVYTLPPSRDELTKNQVSLTCLVKGFYPSDIAVEWESNGQPENNYKTTPPVLDSDGSFFLYSKLTVDKSRWQQGNVFSCSVMHEALHNHYTQKSLSLSPG

SEQ ID NO: 10 - protein, 15 aa, synthetic construct
GGGGSGGGGSGGGGS